European Patent Application EP 4 209 600 A1, published July 12, 2023. Title: SYNTHETIC NUCLEIC ACID CONTROL MOLECULES. Applicant: EXACT SCIENCES CORPORATION. Application EP. The sequence listing filed with the application follows.

SEQUENCE LISTING (18 sequences)

SEQ ID NO: 1 - DNA, 154 bp, synthetic construct
  source 1..154: mol_type = other DNA
acattttcattatttttattataaggcctgctgaaaatgactgaatataaacttgtggtagttggagctggtgacgtaggcaagagtgccttgacgatacagctaattcagaatcattttgtggacgaatatgatccaacaatagaggtaaatc

SEQ ID NO: 2 - DNA, 154 bp, synthetic construct
  source 1..154: mol_type = other DNA
gatttacctctattgttggatcatattcgtccacaaaatgattctgaattagctgtatcgtcaaggcactcttgcctacgtcaccagctccaactaccacaagtttatattcagtcattttcagcaggccttataataaaaataatgaaaatgt

SEQ ID NO: 3 - DNA, 154 bp, synthetic construct
  source 1..154: mol_type = other DNA
acattttcattatttttattataaggcctgctgaaaatgactgaatataaacttgtggtagttggagctgctggcgtaggcaagagtgccttgacgatacagctaattcagaatcattttgtggacgaatatgatccaacaatagaggtaaatc

SEQ ID NO: 4 - DNA, 154 bp, synthetic construct
  source 1..154: mol_type = other DNA
gatttacctctattgttggatcatattcgtccacaaaatgattctgaattagctgtatcgtcaaggcactcttgcctacgccagcagctccaactaccacaagtttatattcagtcattttcagcaggccttataataaaaataatgaaaatgt

SEQ ID NO: 5 - DNA, 126 bp, synthetic construct
  source 1..126: mol_type = other DNA
tttgtctctctgactaggtgtctaagacagtgttgtgggtgtaggtactaacactggctcgtgtgacaaggccatgaggctggtgtaaagcggccttggagtgtgtattaagtaggtgcacagtag

SEQ ID NO: 6 - DNA, 126 bp, synthetic construct
  source 1..126: mol_type = other DNA
ctactgtgcacctacttaatacacactccaaggccgctttacaccagcctcatggccttgtcacacgagccagtgttagtacctacacccacaacactgtcttagacacctagtcagagagacaaa

SEQ ID NO: 7 - DNA, 154 bp, synthetic construct
  source 1..154: mol_type = other DNA
acattttcattatttttattataaggcctgctgaaaatgactgaatataaacttgtggtagttggagctggtggcgtaggcaagagtgccttgacgatacagctaattcagaatcattttgtggacgaatatgatccaacaatagaggtaaatc

SEQ ID NO: 8 - DNA, 154 bp, synthetic construct
  source 1..154: mol_type = other DNA
gatttacctctattgttggatcatattcgtccacaaaatgattctgaattagctgtatcgtcaaggcactcttgcctacgccaccagctccaactaccacaagtttatattcagtcattttcagcaggccttataataaaaataatgaaaatgt

SEQ ID NO: 9 - DNA, 126 bp, synthetic construct
  source 1..126: mol_type = other DNA
gggtgtcccccaggctccgcgtcgnggtcccngctngccctccngccngcccacngggcaccccagcngngcagaaggnggaagccangngngagggaccgcggtccgtccgggactagccccagg

SEQ ID NO: 10 - DNA, 126 bp, synthetic construct
  source 1..126: mol_type = other DNA
cctggggctagtcccggacggaccgcggtccctngngngtggcttcngccttctgngnggctggggtgccnggtgggngggngggagggngagnggggacngcgacgcggagcctgggggacaccc

SEQ ID NO: 11 - DNA, 126 bp, synthetic construct
  source 1..126: mol_type = other DNA
cgggctccgtgcgccctcgccccagctggtttggagttcaaccctnggctcngcngcnggctccttgngccttnggagtgtccngcagngacgccgggagccgacgcgccgcgcgggtacctagcc

SEQ ID NO: 12 - DNA, 126 bp, synthetic construct
  source 1..126: mol_type = other DNA
ggctaggtacccgcgcggcgcgtcggctcccggcgtngctgngggacactcngaaggngcaaggagcnggnggnggagcngagggttgaactccaaaccagctggggcgagggcgcacggagcccg

SEQ ID NO: 13 - DNA, 126 bp, synthetic construct
  source 1..126: mol_type = other DNA
gggtgtcccccaggctccgcgtcgcggtccccgctcgccctcccgcccgcccaccgggcaccccagccgcgcagaaggcggaagccacgcgcgagggaccgcggtccgtccgggactagccccagg

SEQ ID NO: 14 - DNA, 126 bp, synthetic construct
  source 1..126: mol_type = other DNA
cctggggctagtcccggacggaccgcggtccctcgcgcgtggcttccgccttctgcgcggctggggtgcccggtgggcgggcgggagggcgagcggggaccgcgacgcggagcctgggggacaccc

SEQ ID NO: 15 - DNA, 126 bp, synthetic construct
  source 1..126: mol_type = other DNA
cgggctccgtgcgccctcgccccagctggtttggagttcaaccctcggctccgccgccggctccttgcgccttcggagtgtcccgcagcgacgccgggagccgacgcgccgcgcgggtacctagcc

SEQ ID NO: 16 - DNA, 126 bp, synthetic construct
  source 1..126: mol_type = other DNA
ggctaggtacccgcgcggcgcgtcggctcccggcgtcgctgcgggacactccgaaggcgcaaggagccggcggcggagccgagggttgaactccaaaccagctggggcgagggcgcacggagcccg

SEQ ID NO: 17 - DNA, 55 bp, synthetic construct
  source 1..55: mol_type = other DNA
gttcaaccctnggctcngcngcnggctccttgngccttnggagtgtccngcagng

SEQ ID NO: 18 - DNA, 55 bp, synthetic construct
  source 1..55: mol_type = other DNA
ngctgngggacactcngaaggngcaaggagcnggnggnggagcngagggttgaac